European Patent Application EP 4 534 549 A1, published April 9, 2025. Title: mreC Mutant and use thereof in production of L-Valine. Applicant: Anhui Huaheng Biotechnology Co.,Ltd. The sequence listing filed with the application follows.

SEQUENCE LISTING (78 sequences)

SEQ ID NO: 1 - DNA, 1104 bp, synthetic construct
  misc_feature 1..1104: note = synthesized
  source 1..1104: mol_type = other DNA
atgaagccaatttttagccgtggcccgtcgctacagattcgccttattctggcggtgctggtggcgctcggcattattattgccgacagccgcctggggacgttcagtcaaatccgtacttatatggataccgccgtcagtcctttctactttgtttccaatgctcctcgtgaattgctggatggcgtatcgcagacgctggcctcgcgtgaccaattagaacttgaaaaccgggcgttacgtcaggaactgttgctgaaaaacagtgaactgctgatgcttggacaatacaaacaggagaacgcgcgtctgcgcgagctgctgggttccccgctgcgtcaggatgagcagaaaatggtgactcaggttatctccacggttaacgatccttatagcgatcaagttgttatcgataaaggtagcgttaatggcgtttatgaaggccagccggtcatcagcgacaaaggtgttgttggtcaggtggtggccgtcgctaaactgaccagtcgcgtgctgctgatttgtgatgcgacccacgcgctgccaatccaggtgctgcgcaacgatatccgcgtaattgcagccggtaacggttgtacggatgatttgcagcttgagcatctgccggcgaatacggatattcgtgttggtgatgtgctggtgacttccggtctgggcggtcgtttcccggaaggctatccggtcgcggttgtctcttccgtaaaactcgatacccagcgcgcttatactgtgattcaggcgcgtccgactgcagggctgcaacgtttgcgttatctgctgctgctgtggggggcagatcgtaacggcgctaacccgatgacgccggaagaggtgcatcgtgttgctaatgaacgtctgatgcagatgatgccgcaggtattgccttcgccagacgcgatggggccaaagttacctgaaccggcaacggggatcgctcagccgactccgcagcaaccggcgacaggaaatgcagctactgcgcctgctgcgccgacacagcctgctgctaatcgctctccacaaagggctacgccgccgcaaagtggtgctcaaccgcctgcgcgtgcgccgggagggcaatag

SEQ ID NO: 2 - protein, 367 aa, synthetic construct
  REGION 1..367: note = synthesized
MKPIFSRGPSLQIRLILAVLVALGIIIADSRLGTFSQIRTYMDTAVSPFYFVSNAPRELLDGVSQTLASRDQLELENRALRQELLLKNSELLMLGQYKQENARLRELLGSPLRQDEQKMVTQVISTVNDPYSDQVVIDKGSVNGVYEGQPVISDKGVVGQVVAVAKLTSRVLLICDATHALPIQVLRNDIRVIAAGNGCTDDLQLEHLPANTDIRVGDVLVTSGLGGRFPEGYPVAVVSSVKLDTQRAYTVIQARPTAGLQRLRYLLLLWGADRNGANPMTPEEVHRVANERLMQMMPQVLPSPDAMGPKLPEPATGIAQPTPQQPATGNAATAPAAPTQPAANRSPQRATPPQSGAQPPARAPGGQ

SEQ ID NO: 3 - protein, 367 aa, synthetic construct
  REGION 1..367: note = synthesized
MKPIFSRGPSLQIRLILAVLVALGIIIADSRLGTFSQIRTYMDTAVSPFYFVSNAPRELLDGVSQTLASRDQLELENRALRQELLLKNSELLMLGQYKQENARLRELLGSPLRQDEQKMVTQVISTVNDPYSDQVVIDKGSVNGVYEGQLVISDKGVVGQVVAVAKLTSRVLLICDATHALPIQVLRNDIRVIAAGNGCTDDLQLEHLPANTDIRVGDVLVTSGLGGRFPEGYPVAVVSSVKLDTQRAYTVIQARPTAGLQRLRYLLLLWGADRNGANPMTPEEVHRVANERLMQMMPQVLPSPDAMGPKLPEPATGIAQPTPQQPATGNAATAPAAPTQPAANRSPQRATPPQSGAQPPARAPGGQ

SEQ ID NO: 4 - DNA, 1104 bp, synthetic construct
  misc_feature 1..1104: note = synthesized
  source 1..1104: mol_type = other DNA
atgaagccaatttttagccgtggcccgtcgctacagattcgccttattctggcggtgctggtggcgctcggcattattattgccgacagccgcctggggacgttcagtcaaatccgtacttatatggataccgccgtcagtcctttctactttgtttccaatgctcctcgtgaattgctggatggcgtatcgcagacgctggcctcgcgtgaccaattagaacttgaaaaccgggcgttacgtcaggaactgttgctgaaaaacagtgaactgctgatgcttggacaatacaaacaggagaacgcgcgtctgcgcgagctgctgggttccccgctgcgtcaggatgagcagaaaatggtgactcaggttatctccacggttaacgatccttatagcgatcaagttgttatcgataaaggtagcgttaatggcgtttatgaaggccagctggtcatcagcgacaaaggtgttgttggtcaggtggtggccgtcgctaaactgaccagtcgcgtgctgctgatttgtgatgcgacccacgcgctgccaatccaggtgctgcgcaacgatatccgcgtaattgcagccggtaacggttgtacggatgatttgcagcttgagcatctgccggcgaatacggatattcgtgttggtgatgtgctggtgacttccggtctgggcggtcgtttcccggaaggctatccggtcgcggttgtctcttccgtaaaactcgatacccagcgcgcttatactgtgattcaggcgcgtccgactgcagggctgcaacgtttgcgttatctgctgctgctgtggggggcagatcgtaacggcgctaacccgatgacgccggaagaggtgcatcgtgttgctaatgaacgtctgatgcagatgatgccgcaggtattgccttcgccagacgcgatggggccaaagttacctgaaccggcaacggggatcgctcagccgactccgcagcaaccggcgacaggaaatgcagctactgcgcctgctgcgccgacacagcctgctgctaatcgctctccacaaagggctacgccgccgcaaagtggtgctcaaccgcctgcgcgtgcgccgggagggcaatag

SEQ ID NO: 5 - DNA, 73 bp, synthetic construct
  misc_feature 1..73: note = synthesized
  source 1..73: mol_type = other DNA
ttcaacatcactggagaaagtcttatgaaactcgccgtttatagcacaaatgtgacggaagatcacttcgcag

SEQ ID NO: 6 - DNA, 75 bp, synthetic construct
  misc_feature 1..75: note = synthesized
  source 1..75: mol_type = other DNA
agcggcaagattaaaccagttcgttcgggcaggtttcgcctttttccagattatttgttaactgttaattgtcct

SEQ ID NO: 7 - DNA, 20 bp, synthetic construct
  misc_feature 1..20: note = synthesized
  source 1..20: mol_type = other DNA
gataacggagatcgggaatg

SEQ ID NO: 8 - DNA, 20 bp, synthetic construct
  misc_feature 1..20: note = synthesized
  source 1..20: mol_type = other DNA
ctttggctgtcagttcacca

SEQ ID NO: 9 - DNA, 71 bp, synthetic construct
  misc_feature 1..71: note = synthesized
  source 1..71: mol_type = other DNA
agcggcaagattaaaccagttcgttcgggcaggtttcgcctttttccagatttgtgctataaacggcgagt

SEQ ID NO: 10 - DNA, 73 bp, synthetic construct
  misc_feature 1..73: note = synthesized
  source 1..73: mol_type = other DNA
aggtacttccatgtcgagtaagttagtactggttctgaactgcggtagtttgtgacggaagatcacttcgcag

SEQ ID NO: 11 - DNA, 75 bp, synthetic construct
  misc_feature 1..75: note = synthesized
  source 1..75: mol_type = other DNA
ggtcggcagaacgctgtaccgctttgtaggtggtgttaccggtgttcagattatttgttaactgttaattgtcct

SEQ ID NO: 12 - DNA, 20 bp, synthetic construct
  misc_feature 1..20: note = synthesized
  source 1..20: mol_type = other DNA
cgggacaacgttcaaaacat

SEQ ID NO: 13 - DNA, 20 bp, synthetic construct
  misc_feature 1..20: note = synthesized
  source 1..20: mol_type = other DNA
attgcccatcttcttgttgg

SEQ ID NO: 14 - DNA, 71 bp, synthetic construct
  misc_feature 1..71: note = synthesized
  source 1..71: mol_type = other DNA
ggtcggcagaacgctgtaccgctttgtaggtggtgttaccggtgttcagaaactaccgcagttcagaacca

SEQ ID NO: 15 - DNA, 72 bp, synthetic construct
  misc_feature 1..72: note = synthesized
  source 1..72: mol_type = other DNA
ctgacgaaacctcgctccggcggggttttttgttatctgcaattcagtactgtgacggaagatcacttcgca

SEQ ID NO: 16 - DNA, 75 bp, synthetic construct
  misc_feature 1..75: note = synthesized
  source 1..75: mol_type = other DNA
tctgcgccggtaaagcgcttacgcgtcgatgttgtgcccgaacttgccatttatttgttaactgttaattgtcct

SEQ ID NO: 17 - DNA, 70 bp, synthetic construct
  misc_feature 1..70: note = synthesized
  source 1..70: mol_type = other DNA
ctgacgaaacctcgctccggcggggttttttgttatctgcaattcagtacttatctctggcggtgttgac

SEQ ID NO: 18 - DNA, 70 bp, synthetic construct
  misc_feature 1..70: note = synthesized
  source 1..70: mol_type = other DNA
tctgcgccggtaaagcgcttacgcgtcgatgttgtgcccgaacttgccatagctgtttcctggtttaaac

SEQ ID NO: 19 - DNA, 22 bp, synthetic construct
  misc_feature 1..22: note = synthesized
  source 1..22: mol_type = other DNA
gttctgcgcggaacacgtatac

SEQ ID NO: 20 - DNA, 20 bp, synthetic construct
  misc_feature 1..20: note = synthesized
  source 1..20: mol_type = other DNA
ccgctacaggccatacagac

SEQ ID NO: 21 - DNA, 72 bp, synthetic construct
  misc_feature 1..72: note = synthesized
  source 1..72: mol_type = other DNA
tgaactaagaggaagggaacaacattcagaccgaaattgaatttttttcatgtgacggaagatcacttcgca

SEQ ID NO: 22 - DNA, 75 bp, synthetic construct
  misc_feature 1..75: note = synthesized
  source 1..75: mol_type = other DNA
ttcacaccctgtgcccgcaacgcatgtaccacccactgtgcgccattcatttatttgttaactgttaattgtcct

SEQ ID NO: 23 - DNA, 70 bp, synthetic construct
  misc_feature 1..70: note = synthesized
  source 1..70: mol_type = other DNA
tgaactaagaggaagggaacaacattcagaccgaaattgaatttttttcattatctctggcggtgttgac

SEQ ID NO: 24 - DNA, 71 bp, synthetic construct
  misc_feature 1..71: note = synthesized
  source 1..71: mol_type = other DNA
ttcacaccctgtgcccgcaacgcatgtaccacccactgtgcgccattcatagctgtttcctggtttaaacg

SEQ ID NO: 25 - DNA, 22 bp, synthetic construct
  misc_feature 1..22: note = synthesized
  source 1..22: mol_type = other DNA
gcataagatatcgctgctgtag

SEQ ID NO: 26 - DNA, 20 bp, synthetic construct
  misc_feature 1..20: note = synthesized
  source 1..20: mol_type = other DNA
gccagttttgccagtagcac

SEQ ID NO: 27 - DNA, 72 bp, synthetic construct
  misc_feature 1..72: note = synthesized
  source 1..72: mol_type = other DNA
agaacctgattatgcgccggatattatcagtcttactcgaaaatgaatcatgtgacggaagatcacttcgca

SEQ ID NO: 28 - DNA, 75 bp, synthetic construct
  misc_feature 1..75: note = synthesized
  source 1..75: mol_type = other DNA
ttcatcgcccacggtctggatggtcatacgcgataatgtcggatcgtcggttatttgttaactgttaattgtcct

SEQ ID NO: 29 - DNA, 74 bp, synthetic construct
  misc_feature 1..74: note = synthesized
  source 1..74: mol_type = other DNA
agaacctgattatgcgccggatattatcagtcttactcgaaaatgaatcagacgcgttattccgcgtgattggc

SEQ ID NO: 30 - DNA, 21 bp, synthetic construct
  misc_feature 1..21: note = synthesized
  source 1..21: mol_type = other DNA
cacaccagagcgagcaacctc

SEQ ID NO: 31 - DNA, 23 bp, synthetic construct
  misc_feature 1..23: note = synthesized
  source 1..23: mol_type = other DNA
atgagctggaaagcaaacttagc

SEQ ID NO: 32 - DNA, 72 bp, synthetic construct
  misc_feature 1..72: note = synthesized
  source 1..72: mol_type = other DNA
ataactctaatgtttaaactcttttagtaaatcacagtgagtgtgagcgctgtgacggaagatcacttcgca

SEQ ID NO: 33 - DNA, 75 bp, synthetic construct
  misc_feature 1..75: note = synthesized
  source 1..75: mol_type = other DNA
ccgtttatgttgccagacagcgctactgattaagcggattttttcgctttttatttgttaactgttaattgtcct

SEQ ID NO: 34 - DNA, 21 bp, synthetic construct
  misc_feature 1..21: note = synthesized
  source 1..21: mol_type = other DNA
catgctaatgtagccaccaaa

SEQ ID NO: 35 - DNA, 20 bp, synthetic construct
  misc_feature 1..20: note = synthesized
  source 1..20: mol_type = other DNA
ttgcaccaccatccagataa

SEQ ID NO: 36 - DNA, 70 bp, synthetic construct
  misc_feature 1..70: note = synthesized
  source 1..70: mol_type = other DNA
ataactctaatgtttaaactcttttagtaaatcacagtgagtgtgagcgcttatctctggcggtgttgac

SEQ ID NO: 37 - DNA, 70 bp, synthetic construct
  misc_feature 1..70: note = synthesized
  source 1..70: mol_type = other DNA
ccgtttatgttgccagacagcgctactgattaagcggattttttcgctttttagataacttttttcttca

SEQ ID NO: 38 - DNA, 73 bp, synthetic construct
  misc_feature 1..73: note = synthesized
  source 1..73: mol_type = other DNA
aaacgaccaccattaatggttgtcgaagtacgcagtaaataaaaaatccatgtgacggaagatcacttcgcag

SEQ ID NO: 39 - DNA, 75 bp, synthetic construct
  misc_feature 1..75: note = synthesized
  source 1..75: mol_type = other DNA
cggtccgaacggcgcgccagcacgacgaccgtctggggtgttacccgtttttatttgttaactgttaattgtcct

SEQ ID NO: 40 - DNA, 70 bp, synthetic construct
  misc_feature 1..70: note = synthesized
  source 1..70: mol_type = other DNA
aaacgaccaccattaatggttgtcgaagtacgcagtaaataaaaaatccattatctctggcggtgttgac

SEQ ID NO: 41 - DNA, 41 bp, synthetic construct
  misc_feature 1..41: note = synthesized
  source 1..41: mol_type = other DNA
gcggaacggtacttaggcattgctgacctcctggtttaaac

SEQ ID NO: 42 - DNA, 41 bp, synthetic construct
  misc_feature 1..41: note = synthesized
  source 1..41: mol_type = other DNA
gtttaaaccaggaggtcagcaatgcctaagtaccgttccgc

SEQ ID NO: 43 - DNA, 74 bp, synthetic construct
  misc_feature 1..74: note = synthesized
  source 1..74: mol_type = other DNA
cggtccgaacggcgcgccagcacgacgaccgtctggggtgttacccgtttttaaccccccagtttcgatttatc

SEQ ID NO: 44 - DNA, 21 bp, synthetic construct
  misc_feature 1..21: note = synthesized
  source 1..21: mol_type = other DNA
ctgcggagccgatctctttac

SEQ ID NO: 45 - DNA, 22 bp, synthetic construct
  misc_feature 1..22: note = synthesized
  source 1..22: mol_type = other DNA
cgagtaataacgtcctgctgct

SEQ ID NO: 46 - DNA, 20 bp, synthetic construct
  misc_feature 1..20: note = synthesized
  source 1..20: mol_type = other DNA
tgcagaaaaccatcgacaag

SEQ ID NO: 47 - DNA, 20 bp, synthetic construct
  misc_feature 1..20: note = synthesized
  source 1..20: mol_type = other DNA
caccaatcagcgtgacaact

SEQ ID NO: 48 - DNA, 72 bp, synthetic construct
  misc_feature 1..72: note = synthesized
  source 1..72: mol_type = other DNA
gaaggcgaatggctgagatgaaaaacctgaaaattgaggtggtgcgctattgtgacggaagatcacttcgca

SEQ ID NO: 49 - DNA, 75 bp, synthetic construct
  misc_feature 1..75: note = synthesized
  source 1..75: mol_type = other DNA
tctcaggctccttaccagtacagggcaacaaacaggattacgatggtggcttatttgttaactgttaattgtcct

SEQ ID NO: 50 - DNA, 70 bp, synthetic construct
  misc_feature 1..70: note = synthesized
  source 1..70: mol_type = other DNA
gaaggcgaatggctgagatgaaaaacctgaaaattgaggtggtgcgctatttatctctggcggtgttgac

SEQ ID NO: 51 - DNA, 77 bp, synthetic construct
  misc_feature 1..77: note = synthesized
  source 1..77: mol_type = other DNA
tctcaggctccttaccagtacagggcaacaaacaggattacgatggtggcttaacggccgttcaaaatatttttttc

SEQ ID NO: 52 - DNA, 73 bp, synthetic construct
  misc_feature 1..73: note = synthesized
  source 1..73: mol_type = other DNA
gtaggaaagttaactacggatgtacattatggaactgacgactcgcactttgtgacggaagatcacttcgcag

SEQ ID NO: 53 - DNA, 75 bp, synthetic construct
  misc_feature 1..75: note = synthesized
  source 1..75: mol_type = other DNA
gcgtttgccacctgtgcaatattacttcagacggtccgcgagataacgctttatttgttaactgttaattgtcct

SEQ ID NO: 54 - DNA, 20 bp, synthetic construct
  misc_feature 1..20: note = synthesized
  source 1..20: mol_type = other DNA
cagctcatcaaccaggtcaa

SEQ ID NO: 55 - DNA, 20 bp, synthetic construct
  misc_feature 1..20: note = synthesized
  source 1..20: mol_type = other DNA
aaaagccgtcacgttattgg

SEQ ID NO: 56 - DNA, 70 bp, synthetic construct
  misc_feature 1..70: note = synthesized
  source 1..70: mol_type = other DNA
gcgtttgccacctgtgcaatattacttcagacggtccgcgagataacgctaagtgcgagtcgtcagttcc

SEQ ID NO: 57 - DNA, 70 bp, synthetic construct
  misc_feature 1..70: note = synthesized
  source 1..70: mol_type = other DNA
gtaggaaagttaactacggatgtacattatggaactgacgactcgcacttttatctctggcggtgttgac

SEQ ID NO: 58 - DNA, 43 bp, synthetic construct
  misc_feature 1..43: note = synthesized
  source 1..43: mol_type = other DNA
gtgtattgaagtagttagccatagctgtttcctggtttaaacc

SEQ ID NO: 59 - DNA, 43 bp, synthetic construct
  misc_feature 1..43: note = synthesized
  source 1..43: mol_type = other DNA
ggtttaaaccaggaaacagctatggctaactacttcaatacac

SEQ ID NO: 60 - DNA, 71 bp, synthetic construct
  misc_feature 1..71: note = synthesized
  source 1..71: mol_type = other DNA
gcgtttgccacctgtgcaatattacttcagacggtccgcgagataacgctttaacccgcaacagcaatacg

SEQ ID NO: 61 - DNA, 72 bp, synthetic construct
  misc_feature 1..72: note = synthesized
  source 1..72: mol_type = other DNA
acaattatcagtctttatccggcgttctaaggtgtttatcccactatcactgtgacggaagatcacttcgca

SEQ ID NO: 62 - DNA, 75 bp, synthetic construct
  misc_feature 1..75: note = synthesized
  source 1..75: mol_type = other DNA
gcaacacgggtttcattggttaaccgttctcttggtatgccaattcgcatttatttgttaactgttaattgtcct

SEQ ID NO: 63 - DNA, 70 bp, synthetic construct
  misc_feature 1..70: note = synthesized
  source 1..70: mol_type = other DNA
acaattatcagtctttatccggcgttctaaggtgtttatcccactatcacttatctctggcggtgttgac

SEQ ID NO: 64 - DNA, 71 bp, synthetic construct
  misc_feature 1..71: note = synthesized
  source 1..71: mol_type = other DNA
gcaacacgggtttcattggttaaccgttctcttggtatgccaattcgcatagctgtttcctggtttaaacg

SEQ ID NO: 65 - DNA, 20 bp, synthetic construct
  misc_feature 1..20: note = synthesized
  source 1..20: mol_type = other DNA
tcatatcacattccttaagc

SEQ ID NO: 66 - DNA, 20 bp, synthetic construct
  misc_feature 1..20: note = synthesized
  source 1..20: mol_type = other DNA
atactttgaacttgttcttt

SEQ ID NO: 67 - DNA, 72 bp, synthetic construct
  misc_feature 1..72: note = synthesized
  source 1..72: mol_type = other DNA
cattcatctcgctaacttcgcttattatggggatcagtttcagggtttcatgtgacggaagatcacttcgca

SEQ ID NO: 68 - DNA, 75 bp, synthetic construct
  misc_feature 1..75: note = synthesized
  source 1..75: mol_type = other DNA
gggtgccgtgggtgtcccacaatgccaatacacttgaaatgattattcatttatttgttaactgttaattgtcct

SEQ ID NO: 69 - DNA, 70 bp, synthetic construct
  misc_feature 1..70: note = synthesized
  source 1..70: mol_type = other DNA
cattcatctcgctaacttcgcttattatggggatcagtttcagggtttcattatctctggcggtgttgac

SEQ ID NO: 70 - DNA, 70 bp, synthetic construct
  misc_feature 1..70: note = synthesized
  source 1..70: mol_type = other DNA
gggtgccgtgggtgtcccacaatgccaatacacttgaaatgattattcatagctgtttcctggtttaaac

SEQ ID NO: 71 - DNA, 20 bp, synthetic construct
  misc_feature 1..20: note = synthesized
  source 1..20: mol_type = other DNA
ttcagtacgtcgacgcaggt

SEQ ID NO: 72 - DNA, 20 bp, synthetic construct
  misc_feature 1..20: note = synthesized
  source 1..20: mol_type = other DNA
gtaatcgcatccagagaggg

SEQ ID NO: 73 - DNA, 73 bp, synthetic construct
  misc_feature 1..73: note = synthesized
  source 1..73: mol_type = other DNA
ggaagtgtctgtttaccctgcctggtctgatacgagaatacgcataactttgtgacggaagatcacttcgcag

SEQ ID NO: 74 - DNA, 74 bp, synthetic construct
  misc_feature 1..74: note = synthesized
  source 1..74: mol_type = other DNA
agaataaggcgaatctgtagcgacgggccacggctaaaaattggcttcatttatttgttaactgttaattgtcc

SEQ ID NO: 75 - DNA, 70 bp, synthetic construct
  misc_feature 1..70: note = synthesized
  source 1..70: mol_type = other DNA
ggaagtgtctgtttaccctgcctggtctgatacgagaatacgcataacttatgaagccaatttttagccg

SEQ ID NO: 76 - DNA, 79 bp, synthetic construct
  misc_feature 1..79: note = synthesized
  source 1..79: mol_type = other DNA
tcagtttagcgacggccaccacctgaccaacaacacctttgtcgctgatgaccagctggccttcataaacgccattaac

SEQ ID NO: 77 - DNA, 20 bp, synthetic construct
  misc_feature 1..20: note = synthesized
  source 1..20: mol_type = other DNA
gttctctgatcggtgaagcc

SEQ ID NO: 78 - DNA, 21 bp, synthetic construct
  misc_feature 1..21: note = synthesized
  source 1..21: mol_type = other DNA
ctgcatcagacgttcattagc